European Patent Specification EP 4 396 347 B1, published February 11, 2026. Title: Chimeric complex and therapeutic uses thereof. Applicant: Universita' degli Studi di Torino. The sequence listing filed with the application follows.

SEQUENCE LISTING (28 sequences)

SEQ ID NO: 1 - RNA, 34 nt, synthetic construct
  misc_feature 1..34: note = GL21.T
  source 1..34: mol_type = other RNA
atgatcaatcgcctcaattcgacaggaggctcac

SEQ ID NO: 2 - RNA, 17 nt, synthetic construct
  misc_feature 1..17: note = first adhesive sequence
  source 1..17: mol_type = other RNA
gtacattctagatagcc

SEQ ID NO: 3 - DNA, 64 bp, synthetic construct
  misc_feature 1..64: note = binding sequence with multiple anti-miR-214 sites
  source 1..64: mol_type = other DNA
actgcctgtccatcctgctgtcctcttcatcgtcaaactgcctgtcaaacctgctgtaataccc

SEQ ID NO: 4 - DNA, 17 bp, synthetic construct
  misc_feature 1..17: note = second adhesive sequence
  source 1..17: mol_type = other DNA
ggctatctagaatgtac

SEQ ID NO: 5 - RNA, 34 nt, synthetic construct
  misc_feature 1..34: note = GL21.T scramble
  source 1..34: mol_type = other RNA
ggcgctagaaccttctaagcgaatacattaccgc

SEQ ID NO: 6 - DNA, 81 bp, synthetic construct
  misc_feature 1..81: note = miR-214sponge
  source 1..81: mol_type = other DNA
actgcctgtccatcctgctgtcctcttcatcgtcaaactgcctgtcaaacctgctgtaatacccggctatctagaatgtac

SEQ ID NO: 7 - DNA, 64 bp, synthetic construct
  misc_feature 1..64: note = binding sequence
  source 1..64: mol_type = other DNA
actgcctgtctaacctgctgtaactaccaataccaaactgcctgtcaaccctgctgtcttttgt

SEQ ID NO: 8 - DNA, 64 bp, synthetic construct
  misc_feature 1..64: note = binding sequence
  source 1..64: mol_type = other DNA
actgcctgtccgtcctgctgtcccatctatttccttactgcctgtccaccctgctgtttaatcc

SEQ ID NO: 9 - DNA, 64 bp, synthetic construct
  misc_feature 1..64: note = binding sequence
  source 1..64: mol_type = other DNA
actgcctgtccctcctgctgtaacaaccttcaccgaactgcctgtccatcctgctgtatcatcc

SEQ ID NO: 10 - DNA, 64 bp, synthetic construct
  misc_feature 1..64: note = binding sequence
  source 1..64: mol_type = other DNA
actgcctgtcaatcctgctgtcactaatttcatccaactgcctgtcacccctgctgtctatccc

SEQ ID NO: 11 - DNA, 64 bp, synthetic construct
  misc_feature 1..64: note = binding sequence
  source 1..64: mol_type = other DNA
actgcctgtccgtcctgctgtatcttacttcatcaaactgcctgtccctcctgctgtccccccc

SEQ ID NO: 12 - DNA, 64 bp, synthetic construct
  misc_feature 1..64: note = binding sequence
  source 1..64: mol_type = other DNA
actgcctgtccgtcctgctgtcgtatcctaccttaaactgcctgtcccacctgctgtatccccc

SEQ ID NO: 13 - DNA, 64 bp, synthetic construct
  misc_feature 1..64: note = binding sequence
  source 1..64: mol_type = other DNA
actgcctgtccatcctgctgtcattactccccttatactgcctgtcaatcctgctgttattccc

SEQ ID NO: 14 - DNA, 64 bp, synthetic construct
  misc_feature 1..64: note = binding sequence
  source 1..64: mol_type = other DNA
actgcctgtccatcctgctgtctcccgtttctttttactgcctgtccctcctgctgtcgtctcc

SEQ ID NO: 15 - DNA, 64 bp, synthetic construct
  misc_feature 1..64: note = binding sequence
  source 1..64: mol_type = other DNA
actgcctgtcaatcctgctgtatccttatcgaattaactgcctgtccctcctgctgtcgtcccc

SEQ ID NO: 16 - DNA, 64 bp, synthetic construct
  misc_feature 1..64: note = binding sequence
  source 1..64: mol_type = other DNA
actgcctgtcacccctgctgttttcccatccccattactgcctgtcccacctgctgtctctttt

SEQ ID NO: 17 - DNA, 64 bp, synthetic construct
  misc_feature 1..64: note = binding sequence
  source 1..64: mol_type = other DNA
actgcctgtctatcctgctgttaaaaacctttaaatactgcctgtctcccctgctgttaccatt

SEQ ID NO: 18 - DNA, 64 bp, synthetic construct
  misc_feature 1..64: note = binding sequence
  source 1..64: mol_type = other DNA
actgcctgtctaccctgctgtcctaaaaatttataaactgcctgtccaacctgctgtccccttt

SEQ ID NO: 19 - DNA, 64 bp, synthetic construct
  misc_feature 1..64: note = binding sequence
  source 1..64: mol_type = other DNA
actgcctgtcaaccctgctgtaatctgtgtttatgtactgcctgtcccccctgctgtctcccct

SEQ ID NO: 20 - DNA, 64 bp, synthetic construct
  misc_feature 1..64: note = binding sequence
  source 1..64: mol_type = other DNA
actgcctgtccatcctgctgttttcctttctcatatactgcctgtcaatcctgctgtaatccgt

SEQ ID NO: 21 - DNA, 64 bp, synthetic construct
  misc_feature 1..64: note = binding sequence
  source 1..64: mol_type = other DNA
actgcctgtctatcctgctgtcgtcaaacttatcatactgcctgtccctcctgctgtctaccct

SEQ ID NO: 22 - DNA, 64 bp, synthetic construct
  misc_feature 1..64: note = binding sequence
  source 1..64: mol_type = other DNA
actgcctgtcaaccctgctgtgctcatccctcatcaactgcctgtccctcctgctgtctccaat

SEQ ID NO: 23 - DNA, 64 bp, synthetic construct
  misc_feature 1..64: note = binding sequence
  source 1..64: mol_type = other DNA
actgcctgtcacccctgctgtatttttccaatccgaactgcctgtcacccctgctgtctcttat

SEQ ID NO: 24 - DNA, 64 bp, synthetic construct
  misc_feature 1..64: note = binding sequence
  source 1..64: mol_type = other DNA
actgcctgtccatcctgctgtgtcttaactcccataactgcctgtccatcctgctgtaaccttt

SEQ ID NO: 25 - DNA, 64 bp, synthetic construct
  misc_feature 1..64: note = binding sequence
  source 1..64: mol_type = other DNA
actgcctgtcaaacctgctgtccacccactaaacctactgcctgtccatcctgctgtaataatt

SEQ ID NO: 26 - DNA, 64 bp, synthetic construct
  misc_feature 1..64: note = binding sequence
  source 1..64: mol_type = other DNA
actgcctgtcaatcctgctgtactcaaataaataatactgcctgtcaatcctgctgttcctcgt

SEQ ID NO: 27 - DNA, 64 bp, synthetic construct
  misc_feature 1..64: note = binding sequence
  source 1..64: mol_type = other DNA
actgcctgtcaatcctgctgttttaccctcacaattactgcctgtcaaccctgctgtcaataat

SEQ ID NO: 28 - DNA, 64 bp, synthetic construct
  misc_feature 1..64: note = binding sequence
  source 1..64: mol_type = other DNA
actgcctgtcaaccctgctgtacctctcacctatcaactgcctgtcccccctgctgtctaccgt